European Patent Specification EP 4 244 376 B1, published June 18, 2025. Title: Methods and constructs for locating and profiling single cells in a biological sample Name. Applicant: SCellex Oy. The sequence listing filed with the application follows.

SEQUENCE LISTING (33 sequences)

SEQ ID NO: 1 - DNA, 60 bp, Artificial Sequence
  Oligonucleotide
ccttggcacccgagaattccaatcacgbaaaaaaaaaaaaaaaaaaaaaaaaaaaaaaaa

SEQ ID NO: 2 - DNA, 60 bp, Artificial Sequence
  Oligonucleotide
ccttggcacccgagaattccattaggcbaaaaaaaaaaaaaaaaaaaaaaaaaaaaaaaa

SEQ ID NO: 3 - DNA, 60 bp, Artificial Sequence
  Oligonucleotide
ccttggcacccgagaattccatgaccabaaaaaaaaaaaaaaaaaaaaaaaaaaaaaaaa

SEQ ID NO: 4 - DNA, 60 bp, Artificial Sequence
  Oligonucleotide
ccttggcacccgagaattccaacagtgbaaaaaaaaaaaaaaaaaaaaaaaaaaaaaaaa

SEQ ID NO: 5 - DNA, 60 bp, Artificial Sequence
  Oligonucleotide
ccttggcacccgagaattccagccaatbaaaaaaaaaaaaaaaaaaaaaaaaaaaaaaaa

SEQ ID NO: 6 - DNA, 60 bp, Artificial Sequence
  Oligonucleotide
ccttggcacccgagaattccacagatcbaaaaaaaaaaaaaaaaaaaaaaaaaaaaaaaa

SEQ ID NO: 7 - DNA, 60 bp, Artificial Sequence
  Oligonucleotide
ccttggcacccgagaattccaacttgabaaaaaaaaaaaaaaaaaaaaaaaaaaaaaaaa

SEQ ID NO: 8 - DNA, 60 bp, Artificial Sequence
  Oligonucleotide
ccttggcacccgagaattccatgaacgbaaaaaaaaaaaaaaaaaaaaaaaaaaaaaaaa

SEQ ID NO: 9 - DNA, 60 bp, Artificial Sequence
  Oligonucleotide
ccttggcacccgagaattccactgagabaaaaaaaaaaaaaaaaaaaaaaaaaaaaaaaa

SEQ ID NO: 10 - DNA, 60 bp, Artificial Sequence
  Oligonucleotide
ccttggcacccgagaattccatagctgbaaaaaaaaaaaaaaaaaaaaaaaaaaaaaaaa

SEQ ID NO: 11 - DNA, 60 bp, Artificial Sequence
  Oligonucleotide
ccttggcacccgagaattccaaatacgbaaaaaaaaaaaaaaaaaaaaaaaaaaaaaaaa

SEQ ID NO: 12 - DNA, 60 bp, Artificial Sequence
  Oligonucleotide
ccttggcacccgagaattccattccagbaaaaaaaaaaaaaaaaaaaaaaaaaaaaaaaa

SEQ ID NO: 13 - DNA, 60 bp, Artificial Sequence
  Oligonucleotide
ccttggcacccgagaattccaatctgtbaaaaaaaaaaaaaaaaaaaaaaaaaaaaaaaa

SEQ ID NO: 14 - DNA, 60 bp, Artificial Sequence; identical to SEQ ID NO: 7
  Oligonucleotide

SEQ ID NO: 15 - DNA, 60 bp, Artificial Sequence
  Oligonucleotide
ccttggcacccgagaattccataacagbaaaaaaaaaaaaaaaaaaaaaaaaaaaaaaaa

SEQ ID NO: 16 - DNA, 60 bp, Artificial Sequence
  Oligonucleotide
ccttggcacccgagaattccagatgtgbaaaaaaaaaaaaaaaaaaaaaaaaaaaaaaaa

SEQ ID NO: 17 - DNA, 82 bp, Artificial Sequence
  Oligonucleotide
  misc_feature 33..44: /note="a barcode sequence slot for a variable cell barcode , each n can be a, c, g or t "
  misc_feature 45..52: /note="a barcode sequence slot for unique molecular barcode "UMB" , each n can be a, c, g or t "
tttttttaagcagtggtatcaacgcagagtacnnnnnnnnnnnnnnnnnnnntttttttttttttttttttttttttttttt

SEQ ID NO: 18 - DNA, 30 bp, Artificial Sequence
  /note="combined DNA/RNA molecule" /note="Oligonucleotide"
  misc_RNA 28..30
aagcagtggtatcaacgcagagtgaatggg

SEQ ID NO: 19 - DNA, 23 bp, Artificial Sequence
  Oligonucleotide
aagcagtggtatcaacgcagagt

SEQ ID NO: 20 - DNA, 66 bp, Artificial Sequence
  /note="combined DNA/RNA molecule" /note="Oligonucleotide"
  misc_RNA 64..66
aatgatacggcgaccaccgagatctacacgcctgtccgcggaagcagtggtatcaacgcagagtac

SEQ ID NO: 21 - DNA, 37 bp, Artificial Sequence
  Oligonucleotide
gcctgtccgcggaagcagtggtatcaacgcagagtac

SEQ ID NO: 22 - DNA, 10 bp, Artificial Sequence
  Oligonucleotide
cccccccccc

SEQ ID NO: 23 - DNA, 10 bp, Artificial Sequence
  Oligonucleotide
cccccccccc

SEQ ID NO: 24 - DNA, 10 bp, Artificial Sequence
  Oligonucleotide
cccccccccc

SEQ ID NO: 25 - DNA, 10 bp, Artificial Sequence
  Oligonucleotide
cccccccccc

SEQ ID NO: 26 - DNA, 20 bp, Artificial Sequence
  /note="combined DNA/RNA molecule" /note="Oligonucleotide"
  misc_RNA 18..20
ccttggcacccgagaattcc

SEQ ID NO: 27 - DNA, 63 bp, Artificial Sequence
  Oligonucleotide
caagcagaagacggcatacgagatcgtgatgtgactggagttccttggcacccgagaattcca

SEQ ID NO: 28 - DNA, 88 bp, Artificial Sequence
  Oligonucleotide
  misc_feature 33..38: /note="an optional colour tagging sequence slot, each n can be a, c, g or t "
  misc_feature 51..58: /note="a sequence slot for barcodes in oligonucleotides used with ColourBC beads, each n can be a, c, g or t "
tttttttaagcagtggtatcaacgcagagtacnnnnnnbcbcbcbcbcbcnnnnnnnntttttttttttttttttttttttttttttt

SEQ ID NO: 29 - DNA, 10 bp, Artificial Sequence
  Oligonucleotide (partial sequence)
tttttttttt

SEQ ID NO: 30 - DNA, 10 bp, Artificial Sequence
  Oligonucleotide (partial sequence)
aaaaaaaaaa

SEQ ID NO: 31 - DNA, 32 bp, Artificial Sequence
  Oligonucleotide
tttttttaagcagtggtatcaacgcagagtac

SEQ ID NO: 32 - DNA, 30 bp, Artificial Sequence
  Oligonucleotide
aaaaaaaaaaaaaaaaaaaaaaaaaaaaaa

SEQ ID NO: 33 - DNA, 67 bp, Artificial Sequence
  Oligonucleotide
  misc_feature 31..42: /note="unique molecular barcode, UMB, each n can be a, c, g or t "
aaaaaaaaaaaaaaaaaaaaaaaaaaaaaannnnnnnnnnnngtactctgcgttgataccactgctt